European Patent Specification EP 3 274 052 B1, published January 14, 2026. Title: HISTAMINE-PRODUCING BACTERIAL STRAINS AND THEIR USE IN CANCER. Applicant: BIOGAIA AB. The sequence listing filed with the application follows.

SEQUENCE LISTING (25 sequences)

SEQ ID NO: 1 - DNA, 22 bp, Artificial Sequence
  Forward IL-1alpha primer for gene expression studies
cagagagggagtcaactcattg

SEQ ID NO: 2 - DNA, 21 bp, Artificial Sequence
  Reverse IL-1alpha primer for gene expression studies
gtttctggcaactccttcagc

SEQ ID NO: 3 - DNA, 20 bp, Artificial Sequence
  Forward KC primer for gene expression studies
gactccagccacactccaac

SEQ ID NO: 4 - DNA, 18 bp, Artificial Sequence
  Reverse KC primer for gene expression studies
tgacagcgcagctcattg

SEQ ID NO: 5 - DNA, 20 bp, Artificial Sequence
  Forward IL-22 primer for gene expression studies
tgacgaccagaacatccaga

SEQ ID NO: 6 - DNA, 20 bp, Artificial Sequence
  Reverse IL-22 primer for gene expression studies
aatcgccttgatctctccac

SEQ ID NO: 7 - DNA, 20 bp, Artificial Sequence
  Forward IL-10 primer for gene expression studies
cagagccacatgctcctaga

SEQ ID NO: 8 - DNA, 20 bp, Artificial Sequence
  Reverse IL-10 primer for gene expression studies
tgtccagctggtcctttgtt

SEQ ID NO: 9 - DNA, 18 bp, Artificial Sequence
  Forward SPDEF primer for gene expression studies
cctcctggtccctgaggt

SEQ ID NO: 10 - DNA, 19 bp, Artificial Sequence
  Reverse SPDEF primer for gene expression studies
cagtgaatgtggccctgac

SEQ ID NO: 11 - DNA, 18 bp, Artificial Sequence
  Forward H2R primer for gene expression studies
taagcgacccggtacagc

SEQ ID NO: 12 - DNA, 22 bp, Artificial Sequence
  Reverse H2R primer for gene expression studies
tcgatggcttaaggtacaacac

SEQ ID NO: 13 - DNA, 20 bp, Artificial Sequence
  Forward GAPDH primer for gene expression studies
gccaaaagggtcatcatctc

SEQ ID NO: 14 - DNA, 20 bp, Artificial Sequence
  Reverse GAPDH primer for gene expression studies
cacacccatcacaaacatgg

SEQ ID NO: 15 - protein, 6 aa, Lactobacillus reuteri
EERNMR

SEQ ID NO: 16 - protein, 11 aa, Lactobacillus reuteri
DVAAGGVLISA

SEQ ID NO: 17 - protein, 7 aa, Lactobacillus reuteri
DKHQTEK

SEQ ID NO: 18 - protein, 13 aa, Lactobacillus reuteri
NMRYHLLAACLAI

SEQ ID NO: 19 - protein, 7 aa, Lactobacillus reuteri
EERNMRY

SEQ ID NO: 20 - protein, 27 aa, Lactobacillus reuteri
KAKDVAAGGVLISAIFSVLVGLIIFIP

SEQ ID NO: 21 - DNA, 22 bp, Artificial Sequence
  Forward dagK primer for PCR
tggactcacgcgataaacatca

SEQ ID NO: 22 - DNA, 24 bp, Artificial Sequence
  Reverse dagK primer for PCR
acaatcaaatctgtaacagcttcg

SEQ ID NO: 23 - DNA, 20 bp, Artificial Sequence
  Forward hdcA primer for PCR
cgtcaytatccwgctccwgg

SEQ ID NO: 24 - DNA, 20 bp, Artificial Sequence
  Reverse hdcA primer for PCR
tccatrtcagtatcwggkgt

SEQ ID NO: 25 - protein, 131 aa, Lactobacillus reuteri
MDSRDKHQTEKNHHLIQAMRHAIDGIIQVLREERNMRYHLLAACLAIIMSALLQISAMEWLWILLAIFVVFTSEFLNTVTEAVTDLIVDHHYELNVKKAKDVAAGGVLISAIFSVLVGLIIFIPRILAIIR